European Patent Application EP 4 624 575 A1, published October 1, 2025. Title: USE OF ANTISENSE OLIGONUCLEOTIDE IN PREPARATION OF DRUG FOR TREATING DISEASE CAUSED BY ABNORMAL THYROID. Applicant: Hangzhou Tianlong Pharmaceutical Co., Ltd. The sequence listing filed with the application follows.

SEQUENCE LISTING (7 sequences)

SEQ ID NO: 1 - DNA, 20 bp, synthetic construct
  source 1..20: mol_type = other DNA
  modified_base 1..19: mod_base = OTHER; note = phosphorothioate bond
tcctccggagccagacttca

SEQ ID NO: 2 - DNA, 20 bp, synthetic construct
  source 1..20: mol_type = other DNA
  modified_base 1..19: mod_base = OTHER; note = phosphorothioate bond
ttcattccttttatttggga

SEQ ID NO: 3 - DNA, 18 bp, synthetic construct
  source 1..18: mol_type = other DNA
  modified_base 1..17: mod_base = OTHER; note = phosphorothioate bond
ggaccctcctccggagcc

SEQ ID NO: 4 - DNA, 20 bp, synthetic construct
  source 1..20: mol_type = other DNA
  modified_base 1..19: mod_base = OTHER; note = phosphorothioate bond
gagaaacaggagcccccaca

SEQ ID NO: 5 - DNA, 20 bp, synthetic construct
  source 1..20: mol_type = other DNA
  modified_base 1..19: mod_base = OTHER; note = phosphorothioate bond
gcgcggctggaaagcgcgtt

SEQ ID NO: 6 - RNA, 20 nt, synthetic construct
  source 1..20: mol_type = other RNA
  modified_base 7: mod_base = OTHER; note = thymine
  modified_base 17: mod_base = OTHER; note = thymine
  modified_base 20: mod_base = OTHER; note = thymine
cacagatagaagggcctcgt

SEQ ID NO: 7 - RNA, 20 nt, synthetic construct
  source 1..20: mol_type = other RNA
  modified_base 6: mod_base = OTHER; note = thymine
  modified_base 12: mod_base = OTHER; note = thymine
  modified_base 15: mod_base = OTHER; note = thymine
ccaggtgaagctactgcaag